European Patent Specification EP 3 626 734 B1, published February 18, 2026. Title: PEPTIDE THAT REGULATES FAT METABOLISM AND METHOD FOR REGULATING FAT METABOLISM. Applicant: Shenzhen Institutes of Advanced Technology. The sequence listing filed with the application follows.

SEQUENCE LISTING (18 sequences)

SEQ ID NO: 1 - protein, 14 aa, Mouse - Mus musculus
YLGASVPSPDPLEP

SEQ ID NO: 2 - protein, 18 aa, Human - Homo sapiens
YLYQWLGAPVPYPDPLEP

SEQ ID NO: 3 - protein, 19 aa, Artificial Sequence
  ISAP3
YLYQWLGAPVPYPDPLEPR

SEQ ID NO: 4 - protein, 18 aa, Rat - Rattus norvegicus
YLNNGLGAPAPYPDPLEP

SEQ ID NO: 5 - protein, 18 aa, Bonobo - Pan troglodytes
YLYQWLGAPVPYPDTLEP

SEQ ID NO: 6 - protein, 18 aa, Macaque - Macaca mulatta
YLYQWLGAPVPYPDPLEP

SEQ ID NO: 7 - protein, 18 aa, Cow - Bos taurus
YLDHWLGAPAPYPDPLEP

SEQ ID NO: 8 - protein, 18 aa, Sheep - Ovis aries
YLDPGLGAPAPYPDPLEP

SEQ ID NO: 9 - protein, 18 aa, Wild boar - Sus scrofa
YLDHGLGAPAPYPDPLEP

SEQ ID NO: 10 - protein, 18 aa, Naked mole rat - Heterocephalus glaber
YLDQGLGAPAPAPDPLEP

SEQ ID NO: 11 - protein, 18 aa, Dog - Canis lupus
YLDSGLGAPVPYPDPLEP

SEQ ID NO: 12 - protein, 10 aa, Human
PVPYPDPLEP

SEQ ID NO: 13 - protein, 8 aa, Human
PYPDPLEP

SEQ ID NO: 14 - protein, 6 aa, Artificial Sequence
  IASP6
PDPLEP

SEQ ID NO: 15 - protein, 10 aa, Mouse
SVPSPDPLEP

SEQ ID NO: 16 - protein, 8 aa, Mouse
PSPDPLEP

SEQ ID NO: 17 - protein, 18 aa, Mouse - Mus musculus
  kind of general formula of ISAP
  misc_feature (3)..(3): Xaa is TyrAsn, Asp or non-exist
  misc_feature (4)..(4): Xaa is Gln, Asn, His, Pro, Ser or non-exist
  misc_feature (5)..(5): Xaa  is Trp, Gly or non-exist
  misc_feature (6)..(6): Xaa is Leu or non-exist
  misc_feature (9)..(9): Xaa is Pro or Se
  misc_feature (10)..(10): Xaa is Ala or Val
  misc_feature (12)..(12): Xaa is Tyr or Ser
  misc_feature (15)..(15): Xaa is Thr or Pro
YLXXXXGAXXPXPDXLEP

SEQ ID NO: 18 - protein, 15 aa, Mouse - Mus musculus
YLGASVPSPDPLEPT